European Patent Application EP 4 174 182 A1, published May 3, 2023. Title: A gene encoding P450 and use the same. Applicant: Kumiai Chemical Industry Co., Ltd. The sequence listing filed with the application follows.

SEQUENCE LISTING (38 sequences)

SEQ ID NO: 1 - DNA, 1452 bp, Triticum aestivum
  CDS (1)..(1452)
ctgccgccgagccccccggccatcccgttcctcggccacctccacctcctggagaagccgttccatgccgcgctgcgccgcctcgccgcgcgcctcggcccggtcttctcgctgcggctcggctcgcgccgcgccgttgtggtctcctcggcggagtgcgccagggagtgcttcacggagcacgacgtgacgttcgccaaccggccccggttcccctcgcagctgctcgtctccttcgacggcgccgcgctcgtcacgtccagctacggcccgcactggcgcaacctccgccgcgtcgccgccgtgcagctgctctccgcgcaccgcgtcgcctgcatgtctggcgtcatcgccggcgaggtgcgcgccatggcgcgccggctgttccgcgccgccgcggcgtcccccggcggcgatggcgccgcgcgggtccagctgaagcggaggctcttcgagctctccctcagcgtgctcatggagaccatcgcccagaccaaggcgacccggtcggaggccgacgccgacacggacatgtccgtggaggcccaggagttcaagaaggtggtggacgagctcatcccgtacctcggcgccgccaacacgtgggattacctgccggtgttgcggtggttcgacgtgttcggcgtgaggaacaagatcctggccgccgtgagcaggagggacgccttcatgctgcgtctcatcgacaacgagcgccggaggctcgacgacgctggcaccgaaggcgacaagaagagcatgatcgccgtgctcctcaatctgcagaagacggagccggaggtgtacgccgataccatgatcacggctctctgcgcgaatttatttggggccggaacggagaccacgtcgacgacgacggagtgggcgatgtcgctgctgctgaaccacccggcggcgctcaaaaaggcgcaggccgagatcgacgcggccgtgggcacctcccggctggtgaccgccgacgacgtgccacggctggcctacctgcagtgcatcgtgagcgagacgctgcggctgtatccggcggcgccgatgctgctgccgcacgagtcctcggcagactgcaaggtgggcggctacaacgtgccgagcggcacgatgctgatggtgaacgcgtacgccatccaccgggacccggcggcgtgggagcggccgctggagttcgtcccggagcggttcgaggacgggaaggccgaggggcggttcatgatcccgttcgggatgggccgccggcggtgccccggggagacgctggcgctgcggaccatcggcatggtgctggccacgctggtgcagtgcttcgactgggagcgcgtcgacggcgcggaggtggacatgacggagggcggcgggctcaccatccccaaggtcgtgccactcgaggccgtgtgcaggccgcgcccggccatgcgcgacgtgcttcagagcctctga

SEQ ID NO: 2 - protein, 483 aa, Triticum aestivum
LPPSPPAIPFLGHLHLLEKPFHAALRRLAARLGPVFSLRLGSRRAVVVSSAECARECFTEHDVTFANRPRFPSQLLVSFDGAALVTSSYGPHWRNLRRVAAVQLLSAHRVACMSGVIAGEVRAMARRLFRAAAASPGGDGAARVQLKRRLFELSLSVLMETIAQTKATRSEADADTDMSVEAQEFKKVVDELIPYLGAANTWDYLPVLRWFDVFGVRNKILAAVSRRDAFMLRLIDNERRRLDDAGTEGDKKSMIAVLLNLQKTEPEVYADTMITALCANLFGAGTETTSTTTEWAMSLLLNHPAALKKAQAEIDAAVGTSRLVTADDVPRLAYLQCIVSETLRLYPAAPMLLPHESSADCKVGGYNVPSGTMLMVNAYAIHRDPAAWERPLEFVPERFEDGKAEGRFMIPFGMGRRRCPGETLALRTIGMVLATLVQCFDWERVDGAEVDMTEGGGLTIPKVVPLEAVCRPRPAMRDVLQSL

SEQ ID NO: 3 - DNA, 1452 bp, Triticum aestivum
  CDS (1)..(1452)
ctgccgccgagcccccaggccatcccgttcctcggccacctccacctcctggagaagccgttccacgccgctctgtgccgcctcgccgagcgcctcggcccggtcttctcgctgcgcctcggctcgcgccgcgccgtggtcgtctcctcggcggagtgcgccagggagtgcttcacggagcacgacgtgatcttcgccgaccggccccagttcccctcgcagctgctcgtgtccttcgacggcatcgcgctctccacgtccagctacggcccgcactggcgcaacctccgccgcgtcgccgccgtgcagctgctctctgcgcaccgcgtcgcctgcatgtccggcgtgatcgggggcgaggtgcgcgccatggcgcgccggctcttccgcgccgccgcggcgtcccccggtggggacggcgccgcgcgggtccagctgaagcggaggctcttcgagctctccctcagcgtgctcatggaaaccatcgcccagaccaaggcgacccggtcggaggccgacgccgacacggacatgtcagaggaggcccaggagttcaagaaggtggtggacgagctcatcccgtacctcggcgccgccaacacgtgggattacctgccggtgttgcggtggttcgacgtgttcggcgtgaggaacaagatcctggccgccgtgagcaggagggacgccttcctgcatcgtctcatcgacaacgagcgccggaggctcgacaacgccggcaccgaaggcgacaagaagagcatgatcgccgtgctcctcaatctgcagaagacggagccggaggtgtacaccgataccatgatcacggctctctgcgcgaatttattcggggccggaacggagaccacgtcgacgacgacggagtgggcgatgtcgctgctgctgaaccacccggcggcgctgaggaaggcgcaggccgagatcgacgcggccgtggggacctcccggctggtgaccgccgacgacgtgccccggctggcctacctgcagtgcatcgtgagcgagacgctgcggctgtacccggcggcgccgatgctgctgccgcaccagtcctcggcggactgcaaggtcggcggctacaacgtgccgagcggcacgatgctgatggtgaacgcgtacgccatccaccgggacccggcggcgtgggagcggccgctggagttcgtcccggagcggttcgagaacgggaaggccgaggggcggttcatgatcccgttcgggatgggccggcggcggtgccccggggagacgctggcgctgcggaccattggcatggtgctggccacgctggtgcagtgcttcgactgggagcgcgtggacggcgcggaggtggacatgacggagggcggagggctcaccatccccaaggtcgtgccgctcgaggccgtgtgcaggccgcgcccggccatgcgcgacgtgcttcagagcctctga

SEQ ID NO: 4 - protein, 483 aa, Triticum aestivum
LPPSPQAIPFLGHLHLLEKPFHAALCRLAERLGPVFSLRLGSRRAVVVSSAECARECFTEHDVIFADRPQFPSQLLVSFDGIALSTSSYGPHWRNLRRVAAVQLLSAHRVACMSGVIGGEVRAMARRLFRAAAASPGGDGAARVQLKRRLFELSLSVLMETIAQTKATRSEADADTDMSEEAQEFKKVVDELIPYLGAANTWDYLPVLRWFDVFGVRNKILAAVSRRDAFLHRLIDNERRRLDNAGTEGDKKSMIAVLLNLQKTEPEVYTDTMITALCANLFGAGTETTSTTTEWAMSLLLNHPAALRKAQAEIDAAVGTSRLVTADDVPRLAYLQCIVSETLRLYPAAPMLLPHQSSADCKVGGYNVPSGTMLMVNAYAIHRDPAAWERPLEFVPERFENGKAEGRFMIPFGMGRRRCPGETLALRTIGMVLATLVQCFDWERVDGAEVDMTEGGGLTIPKVVPLEAVCRPRPAMRDVLQSL

SEQ ID NO: 5 - DNA, 1446 bp, Hordeum vulgare
  CDS (1)..(1446)
ctgccgccgagccccccggccgtcccgttcttcggccacctccacctcgtggagaagccgttgcacgccgcactgtgccgcctcggggcgcgccatgggccggtcttctcgcttcggctcggcgcgcgcaacgccgtggtggtgtcctcgccggcgtgcgccagggagtgcttcacggaccacgacgtggccttcgccaaccggccccagttcccctcgcagatgctcgtgtcctacggcggcacctcgctcgtcagctccagctacggcccgcactggcgcaacctccgccgcgtcgccgccgtgcgcctgctctccgcgcatcgcgtcgccggcatgtcgggcgtcatcgccgccgaggtgcgcgccatggcgcgccgtctgtaccgcgccgccgcggcgtcccccggcggcgccgcgcgcgtggagctcaagcggagcctgttcgagctctccctgagcgtgctcatggagactatcgcgcggaccaagggcacccgctcggaggcggacgccgacacggacatgtcgctggaggcgcaggagttcaagcaggtggtggacgagatcatcccgctcatcggcgcggccaacctgtgggactacctgccggtgatgcggtggttcgacgtgtccggcgtgaggagcaggatcctggccacggtgagcaggagggacgccttcctccaccggctcattgacgccgagcggcggaggatggaagagggcggcgacgagggcgagaagaagagcatgattgccgtgctcctcactctgcaaaagacggagccggagctgtacactgatcagatgatcatcgctctgtgtgcgaatatgtttgtggccggaacagagaccacctcaaccacgatagaatgggcgatgtcgctgctgctgaaccacccggcggcgctcaagaaggcccaggccgagatcgacgcgtccatcgggacctcccgcatggttgccgccgacgacgtgccccgcctcagctacctccagtgcatcatcaacgagacgctacgcatgtacccggcggcgccgctgctgctgccgcacgagtcctccgccgactgcaaggtcggcggctacgacgtgccgagcggcaccatgctgatcgtgaacgcgtacgccatccacagggacccggcgacgtgggaggacccgacggcgttccggccggagcggttcgaggacggcaagggcgacgggctgctgctgatgccgttcgggatggggcggcggaggtgccccggcgaggcgctggcgctgcagacggtcggggttgttctcgggatgctggtgcagtgcttcgactgggatcgggtggacggcgtggaggtggacatgacggagggggtggggatcaccatgcccaagtccgtggctttggaggccgtgtgtaggccgcgtgctgccatgcgcgatgtccttcacaagctgtga

SEQ ID NO: 6 - protein, 481 aa, Hordeum vulgare
LPPSPPAVPFFGHLHLVEKPLHAALCRLGARHGPVFSLRLGARNAVVVSSPACARECFTDHDVAFANRPQFPSQMLVSYGGTSLVSSSYGPHWRNLRRVAAVRLLSAHRVAGMSGVIAAEVRAMARRLYRAAAASPGGAARVELKRSLFELSLSVLMETIARTKGTRSEADADTDMSLEAQEFKQVVDEIIPLIGAANLWDYLPVMRWFDVSGVRSRILATVSRRDAFLHRLIDAERRRMEEGGDEGEKKSMIAVLLTLQKTEPELYTDQMIIALCANMFVAGTETTSTTIEWAMSLLLNHPAALKKAQAEIDASIGTSRMVAADDVPRLSYLQCIINETLRMYPAAPLLLPHESSADCKVGGYDVPSGTMLIVNAYAIHRDPATWEDPTAFRPERFEDGKGDGLLLMPFGMGRRRCPGEALALQTVGVVLGMLVQCFDWDRVDGVEVDMTEGVGITMPKSVALEAVCRPRAAMRDVLHKL

SEQ ID NO: 7 - DNA, 1452 bp, Hordeum vulgare
  CDS (1)..(1452)
ctgccgccgagccccaggcccatcccgttcctcggccacctccacctcctggagaagccgttccacgtcgctctgtgccgcctcgccgcgcgcctcggcccggtcttctcgctgcggctcggctcgcgccgcgccgtggtggtgtcctcggcggactgcgccagggagtgcttcacggagcacgacgtgatcttcgccaacaggccccagttcccctcgcagctgctcgtgtccttcgacggcaccgcgctctccacgtccagctacggcccgcactggcgcaacctccgtcgcgtcgccgccgtgcagctgctctccgcgcaccgcgtcgcctgcatgtccggcgtcatcgccggcgaggtgcgcgccatggcccgccggctcttccgctccgccgaggcgtcccccggcggcggtggcgccgcgcgggtccagctgaagcggaggctgttcgagctctcattgagcgtgctcatggagaccatcgctcagaccaaggggacccggtcggaggccgacgccgacacggacatgtccgtggaggcccaggagttcaagaaggtggtggacgagatcatcccgtacctcggcgccgccaacacgtgggactacctgccggtggtgcggtggttcgacgtgttcggcgtcaggaacaagatcctggccgccgtgagcaggagggacgccttcctccatcgtctcatcgacgccgagcggaggaggctggacggcggcggcgccgaagccgacaagaagagcatgatcgccgtgctgctcactctgcagaagacggagccggaggtgtacaccgatactatgatcacggctctctgctcgaatttatttggggccggaacggagaccacgtcgacgacgacggagtgggccatgtcgctgcttctgaaccacccggcggcgctgaggaaggcgcaggccgagatcgacgcggccgtgggcacctcccggctggtgaccgccgacgacgtgccccggctcgcctacctgcagtgcatcgtgagcgagacgctgcggctgtacccggcgacgccgatgctgctgccgcaccaatcgtcggcggactgcaaggtgggcggctacaacgtgccgagcggcacgatgctgatggtgaacgcgtacgccatccaccgcgacccggcggcgtgggagcggccgctggagttcgtcccggagcggttcgaggacggcaaggccgaggggcggttcatgatcccgttcgggatgggccgccggcggtgccccggggagacgctggcgctgcggaccatcggcatggtgctggccacgctggtgcagtgcttcgactgggaccgcgtcgacggcaaggaggtggacatgacggagagcggcgggctcaccatccccaaggccgtgccgctcgaggccgtctgcaggccgcgcgcggccatgcgcgacgtgctccagagcctctga

SEQ ID NO: 8 - protein, 483 aa, Hordeum vulgare
LPPSPRPIPFLGHLHLLEKPFHVALCRLAARLGPVFSLRLGSRRAVVVSSADCARECFTEHDVIFANRPQFPSQLLVSFDGTALSTSSYGPHWRNLRRVAAVQLLSAHRVACMSGVIAGEVRAMARRLFRSAEASPGGGGAARVQLKRRLFELSLSVLMETIAQTKGTRSEADADTDMSVEAQEFKKVVDEIIPYLGAANTWDYLPVVRWFDVFGVRNKILAAVSRRDAFLHRLIDAERRRLDGGGAEADKKSMIAVLLTLQKTEPEVYTDTMITALCSNLFGAGTETTSTTTEWAMSLLLNHPAALRKAQAEIDAAVGTSRLVTADDVPRLAYLQCIVSETLRLYPATPMLLPHQSSADCKVGGYNVPSGTMLMVNAYAIHRDPAAWERPLEFVPERFEDGKAEGRFMIPFGMGRRRCPGETLALRTIGMVLATLVQCFDWDRVDGKEVDMTESGGLTIPKAVPLEAVCRPRAAMRDVLQSL

SEQ ID NO: 9 - DNA, 1551 bp, Triticum aestivum
  CDS (1)..(1551)
atggataaggcgtacattgccatcctcaccatcgccttcctcttcctgatccactacgttctgggcaatggccggcgcggcggcaagggcgccgcgcagctgccgccgagccccccggccatcccgttcctcggccacctccacctcctggagaagccgttccatgccgcgctgcgccgcctcgccgcgcgcctcggcccggtcttctcgctgcggctcggctcgcgccgcgccgttgtggtctcctcggcggagtgcgccagggagtgcttcacggagcacgacgtgacgttcgccaaccggccccggttcccctcgcagctgctcgtctccttcgacggcgccgcgctcgtcacgtccagctacggcccgcactggcgcaacctccgccgcgtcgccgccgtgcagctgctctccgcgcaccgcgtcgcctgcatgtctggcgtcatcgccggcgaggtgcgcgccatggcgcgccggctgttccgcgccgccgcggcgtcccccggcggcgatggcgccgcgcgggtccagctgaagcggaggctcttcgagctctccctcagcgtgctcatggagaccatcgcccagaccaaggcgacccggtcggaggccgacgccgacacggacatgtccgtggaggcccaggagttcaagaaggtggtggacgagctcatcccgtacctcggcgccgccaacacgtgggattacctgccggtgttgcggtggttcgacgtgttcggcgtgaggaacaagatcctggccgccgtgagcaggagggacgccttcatgctgcgtctcatcgacaacgagcgccggaggctcgacgacgctggcaccgaaggcgacaagaagagcatgatcgccgtgctcctcaatctgcagaagacggagccggaggtgtacgccgataccatgatcacggctctctgcgcgaatttatttggggccggaacggagaccacgtcgacgacgacggagtgggcgatgtcgctgctgctgaaccacccggcggcgctcaaaaaggcgcaggccgagatcgacgcggccgtgggcacctcccggctggtgaccgccgacgacgtgccacggctggcctacctgcagtgcatcgtgagcgagacgctgcggctgtatccggcggcgccgatgctgctgccgcacgagtcctcggcagactgcaaggtgggcggctacaacgtgccgagcggcacgatgctgatggtgaacgcgtacgccatccaccgggacccggcggcgtgggagcggccgctggagttcgtcccggagcggttcgaggacgggaaggccgaggggcggttcatgatcccgttcgggatgggccgccggcggtgccccggggagacgctggcgctgcggaccatcggcatggtgctggccacgctggtgcagtgcttcgactgggagcgcgtcgacggcgcggaggtggacatgacggagggcggcgggctcaccatccccaaggtcgtgccactcgaggccgtgtgcaggccgcgcccggccatgcgcgacgtgcttcagagcctctga

SEQ ID NO: 10 - protein, 516 aa, Triticum aestivum
MDKAYIAILTIAFLFLIHYVLGNGRRGGKGAAQLPPSPPAIPFLGHLHLLEKPFHAALRRLAARLGPVFSLRLGSRRAVVVSSAECARECFTEHDVTFANRPRFPSQLLVSFDGAALVTSSYGPHWRNLRRVAAVQLLSAHRVACMSGVIAGEVRAMARRLFRAAAASPGGDGAARVQLKRRLFELSLSVLMETIAQTKATRSEADADTDMSVEAQEFKKVVDELIPYLGAANTWDYLPVLRWFDVFGVRNKILAAVSRRDAFMLRLIDNERRRLDDAGTEGDKKSMIAVLLNLQKTEPEVYADTMITALCANLFGAGTETTSTTTEWAMSLLLNHPAALKKAQAEIDAAVGTSRLVTADDVPRLAYLQCIVSETLRLYPAAPMLLPHESSADCKVGGYNVPSGTMLMVNAYAIHRDPAAWERPLEFVPERFEDGKAEGRFMIPFGMGRRRCPGETLALRTIGMVLATLVQCFDWERVDGAEVDMTEGGGLTIPKVVPLEAVCRPRPAMRDVLQSL

SEQ ID NO: 11 - DNA, 1557 bp, Triticum aestivum
  CDS (1)..(1557)
atggataaggcatatatcgccatcctctccttcgccttcctcttcctgctccactacattctaggcaaggtcagcaatggcaggcgcagcaagggcgccgtccagctgccgccgagcccccaggccatcccgttcctcggccacctccacctcctggagaagccgttccacgccgctctgtgccgcctcgccgagcgcctcggcccggtcttctcgctgcgcctcggctcgcgccgcgccgtggtcgtctcctcggcggagtgcgccagggagtgcttcacggagcacgacgtgatcttcgccgaccggccccagttcccctcgcagctgctcgtgtccttcgacggcatcgcgctctccacgtccagctacggcccgcactggcgcaacctccgccgcgtcgccgccgtgcagctgctctctgcgcaccgcgtcgcctgcatgtccggcgtgatcgggggcgaggtgcgcgccatggcgcgccggctcttccgcgccgccgcggcgtcccccggtggggacggcgccgcgcgggtccagctgaagcggaggctcttcgagctctccctcagcgtgctcatggaaaccatcgcccagaccaaggcgacccggtcggaggccgacgccgacacggacatgtcagaggaggcccaggagttcaagaaggtggtggacgagctcatcccgtacctcggcgccgccaacacgtgggattacctgccggtgttgcggtggttcgacgtgttcggcgtgaggaacaagatcctggccgccgtgagcaggagggacgccttcctgcatcgtctcatcgacaacgagcgccggaggctcgacaacgccggcaccgaaggcgacaagaagagcatgatcgccgtgctcctcaatctgcagaagacggagccggaggtgtacaccgataccatgatcacggctctctgcgcgaatttattcggggccggaacggagaccacgtcgacgacgacggagtgggcgatgtcgctgctgctgaaccacccggcggcgctgaggaaggcgcaggccgagatcgacgcggccgtggggacctcccggctggtgaccgccgacgacgtgccccggctggcctacctgcagtgcatcgtgagcgagacgctgcggctgtacccggcggcgccgatgctgctgccgcaccagtcctcggcggactgcaaggtcggcggctacaacgtgccgagcggcacgatgctgatggtgaacgcgtacgccatccaccgggacccggcggcgtgggagcggccgctggagttcgtcccggagcggttcgagaacgggaaggccgaggggcggttcatgatcccgttcgggatgggccggcggcggtgccccggggagacgctggcgctgcggaccattggcatggtgctggccacgctggtgcagtgcttcgactgggagcgcgtggacggcgcggaggtggacatgacggagggcggagggctcaccatccccaaggtcgtgccgctcgaggccgtgtgcaggccgcgcccggccatgcgcgacgtgcttcagagcctctga

SEQ ID NO: 12 - protein, 518 aa, Triticum aestivum
MDKAYIAILSFAFLFLLHYILGKVSNGRRSKGAVQLPPSPQAIPFLGHLHLLEKPFHAALCRLAERLGPVFSLRLGSRRAVVVSSAECARECFTEHDVIFADRPQFPSQLLVSFDGIALSTSSYGPHWRNLRRVAAVQLLSAHRVACMSGVIGGEVRAMARRLFRAAAASPGGDGAARVQLKRRLFELSLSVLMETIAQTKATRSEADADTDMSEEAQEFKKVVDELIPYLGAANTWDYLPVLRWFDVFGVRNKILAAVSRRDAFLHRLIDNERRRLDNAGTEGDKKSMIAVLLNLQKTEPEVYTDTMITALCANLFGAGTETTSTTTEWAMSLLLNHPAALRKAQAEIDAAVGTSRLVTADDVPRLAYLQCIVSETLRLYPAAPMLLPHQSSADCKVGGYNVPSGTMLMVNAYAIHRDPAAWERPLEFVPERFENGKAEGRFMIPFGMGRRRCPGETLALRTIGMVLATLVQCFDWERVDGAEVDMTEGGGLTIPKVVPLEAVCRPRPAMRDVLQSL

SEQ ID NO: 13 - DNA, 1557 bp, Hordeum vulgare
  CDS (1)..(1557)
atggataaggcatccattgccgtcctctccttggccttcctcttcctgctccactacattctgggcaagaggagcgatggcaggcgcggcaagggcaagggcgccgtgcagctgccgccgagccccccggccgtcccgttcttcggccacctccacctcgtggagaagccgttgcacgccgcactgtgccgcctcggggcgcgccatgggccggtcttctcgcttcggctcggcgcgcgcaacgccgtggtggtgtcctcgccggcgtgcgccagggagtgcttcacggaccacgacgtggccttcgccaaccggccccagttcccctcgcagatgctcgtgtcctacggcggcacctcgctcgtcagctccagctacggcccgcactggcgcaacctccgccgcgtcgccgccgtgcgcctgctctccgcgcatcgcgtcgccggcatgtcgggcgtcatcgccgccgaggtgcgcgccatggcgcgccgtctgtaccgcgccgccgcggcgtcccccggcggcgccgcgcgcgtggagctcaagcggagcctgttcgagctctccctgagcgtgctcatggagactatcgcgcggaccaagggcacccgctcggaggcggacgccgacacggacatgtcgctggaggcgcaggagttcaagcaggtggtggacgagatcatcccgctcatcggcgcggccaacctgtgggactacctgccggtgatgcggtggttcgacgtgtccggcgtgaggagcaggatcctggccacggtgagcaggagggacgccttcctccaccggctcattgacgccgagcggcggaggatggaagagggcggcgacgagggcgagaagaagagcatgattgccgtgctcctcactctgcaaaagacggagccggagctgtacactgatcagatgatcatcgctctgtgtgcgaatatgtttgtggccggaacagagaccacctcaaccacgatagaatgggcgatgtcgctgctgctgaaccacccggcggcgctcaagaaggcccaggccgagatcgacgcgtccatcgggacctcccgcatggttgccgccgacgacgtgccccgcctcagctacctccagtgcatcatcaacgagacgctacgcatgtacccggcggcgccgctgctgctgccgcacgagtcctccgccgactgcaaggtcggcggctacgacgtgccgagcggcaccatgctgatcgtgaacgcgtacgccatccacagggacccggcgacgtgggaggacccgacggcgttccggccggagcggttcgaggacggcaagggcgacgggctgctgctgatgccgttcgggatggggcggcggaggtgccccggcgaggcgctggcgctgcagacggtcggggttgttctcgggatgctggtgcagtgcttcgactgggatcgggtggacggcgtggaggtggacatgacggagggggtggggatcaccatgcccaagtccgtggctttggaggccgtgtgtaggccgcgtgctgccatgcgcgatgtccttcacaagctgtga

SEQ ID NO: 14 - protein, 518 aa, Hordeum vulgare
MDKASIAVLSLAFLFLLHYILGKRSDGRRGKGKGAVQLPPSPPAVPFFGHLHLVEKPLHAALCRLGARHGPVFSLRLGARNAVVVSSPACARECFTDHDVAFANRPQFPSQMLVSYGGTSLVSSSYGPHWRNLRRVAAVRLLSAHRVAGMSGVIAAEVRAMARRLYRAAAASPGGAARVELKRSLFELSLSVLMETIARTKGTRSEADADTDMSLEAQEFKQVVDEIIPLIGAANLWDYLPVMRWFDVSGVRSRILATVSRRDAFLHRLIDAERRRMEEGGDEGEKKSMIAVLLTLQKTEPELYTDQMIIALCANMFVAGTETTSTTIEWAMSLLLNHPAALKKAQAEIDASIGTSRMVAADDVPRLSYLQCIINETLRMYPAAPLLLPHESSADCKVGGYDVPSGTMLIVNAYAIHRDPATWEDPTAFRPERFEDGKGDGLLLMPFGMGRRRCPGEALALQTVGVVLGMLVQCFDWDRVDGVEVDMTEGVGITMPKSVALEAVCRPRAAMRDVLHKL

SEQ ID NO: 15 - DNA, 1557 bp, Hordeum vulgare
  CDS (1)..(1557)
atggataaggcatacattgccatcctctccttcactttcctcttcctgctccactacattctaggcaaggtcagcaatggcaggcgcagcaagggtgacgtccagctgccgccgagccccaggcccatcccgttcctcggccacctccacctcctggagaagccgttccacgtcgctctgtgccgcctcgccgcgcgcctcggcccggtcttctcgctgcggctcggctcgcgccgcgccgtggtggtgtcctcggcggactgcgccagggagtgcttcacggagcacgacgtgatcttcgccaacaggccccagttcccctcgcagctgctcgtgtccttcgacggcaccgcgctctccacgtccagctacggcccgcactggcgcaacctccgtcgcgtcgccgccgtgcagctgctctccgcgcaccgcgtcgcctgcatgtccggcgtcatcgccggcgaggtgcgcgccatggcccgccggctcttccgctccgccgaggcgtcccccggcggcggtggcgccgcgcgggtccagctgaagcggaggctgttcgagctctcattgagcgtgctcatggagaccatcgctcagaccaaggggacccggtcggaggccgacgccgacacggacatgtccgtggaggcccaggagttcaagaaggtggtggacgagatcatcccgtacctcggcgccgccaacacgtgggactacctgccggtggtgcggtggttcgacgtgttcggcgtcaggaacaagatcctggccgccgtgagcaggagggacgccttcctccatcgtctcatcgacgccgagcggaggaggctggacggcggcggcgccgaagccgacaagaagagcatgatcgccgtgctgctcactctgcagaagacggagccggaggtgtacaccgatactatgatcacggctctctgctcgaatttatttggggccggaacggagaccacgtcgacgacgacggagtgggccatgtcgctgcttctgaaccacccggcggcgctgaggaaggcgcaggccgagatcgacgcggccgtgggcacctcccggctggtgaccgccgacgacgtgccccggctcgcctacctgcagtgcatcgtgagcgagacgctgcggctgtacccggcgacgccgatgctgctgccgcaccaatcgtcggcggactgcaaggtgggcggctacaacgtgccgagcggcacgatgctgatggtgaacgcgtacgccatccaccgcgacccggcggcgtgggagcggccgctggagttcgtcccggagcggttcgaggacggcaaggccgaggggcggttcatgatcccgttcgggatgggccgccggcggtgccccggggagacgctggcgctgcggaccatcggcatggtgctggccacgctggtgcagtgcttcgactgggaccgcgtcgacggcaaggaggtggacatgacggagagcggcgggctcaccatccccaaggccgtgccgctcgaggccgtctgcaggccgcgcgcggccatgcgcgacgtgctccagagcctctga

SEQ ID NO: 16 - protein, 518 aa, Hordeum vulgare
MDKAYIAILSFTFLFLLHYILGKVSNGRRSKGDVQLPPSPRPIPFLGHLHLLEKPFHVALCRLAARLGPVFSLRLGSRRAVVVSSADCARECFTEHDVIFANRPQFPSQLLVSFDGTALSTSSYGPHWRNLRRVAAVQLLSAHRVACMSGVIAGEVRAMARRLFRSAEASPGGGGAARVQLKRRLFELSLSVLMETIAQTKGTRSEADADTDMSVEAQEFKKVVDEIIPYLGAANTWDYLPVVRWFDVFGVRNKILAAVSRRDAFLHRLIDAERRRLDGGGAEADKKSMIAVLLTLQKTEPEVYTDTMITALCSNLFGAGTETTSTTTEWAMSLLLNHPAALRKAQAEIDAAVGTSRLVTADDVPRLAYLQCIVSETLRLYPATPMLLPHQSSADCKVGGYNVPSGTMLMVNAYAIHRDPAAWERPLEFVPERFEDGKAEGRFMIPFGMGRRRCPGETLALRTIGMVLATLVQCFDWDRVDGKEVDMTESGGLTIPKAVPLEAVCRPRAAMRDVLQSL

SEQ ID NO: 17 - DNA, 23 bp, Artificial
  Synthetic DNA
caacctgagacctcaagtgtcac

SEQ ID NO: 18 - DNA, 21 bp, Artificial
  Synthetic DNA
gtactacctggatccacgagc

SEQ ID NO: 19 - DNA, 35 bp, Artificial
  Synthetic DNA
aaggagatatacatatggataaggcgtacattgcc

SEQ ID NO: 20 - DNA, 35 bp, Artificial
  Synthetic DNA
gtggtggtgctcgagtcagaggctctgaagcacgt

SEQ ID NO: 21 - DNA, 2091 bp, Triticum aestivum
atgagggactcggcgctcgacctgctggcggcgctgctcacgggccgggccccgccggccgccgccgacggggaccagaaccgccgcctgctcgcgctgctcgccacctccctcgccgtgctcgtcggctgcggcgtcgcgctcctcttccgccgctcctcctccggcgccgcgccgctcgcccacaagtccgccgcggccaagcccctcgcagcgaagaaggaccaggagcccgaccccgacgacggccgccagcgggtcgccctcttcttcggcacgcagaccggcaccgccgagggcttcgccaaggcgctcgcggaggaggccaaggccaggtacgacaaggccgtcttcaaggtgctcgatctggatgactatgccgcggaggacgaggagtacgaggagaagctcaagaaggagaacatcgccttcttcttcctcgcaacgtatggggacggtgagccaaccgacaatgccgccagattctacaaatggttctccgagggaaacgagaggggtgagtggttgagcaacctcaagttcggggtgtttgctcttgggaataggcagtacgagcatttcaacaaggtcggaaaggaggtcgatcagctcctcgccgaacaaggtggaaagcgcatagttcctgttggccttggagatgacgatcaatgcattgaggatgacttcaatgcctggaaggaactactgtggccagaattggacaaactgctccgcgttgaagataattcttcaacagcacaatctccttacacagctgctattccgcaatatagagttgtgcttaccaaaccagaggatgccacacatatcaacaagtctttcagtcttagcaatggtcatgtcgtctacgacagtcaacatccttgcagggcaaatgtggctgtgcgacgggagcttcacacaccagcttctgaccggtcctgcattcatttggaatttgatattgcaggaactagccttacatatgagactggagatcatgttggtgtgtacgcagaaaattcaattgagactgtagaggaggcagaaaagctattagattattcaccagatacttatttctcaatttatgctgaccaagaggatggcactccactttttgggggctctttgccacctcctttcccatctccctgtactgtgagggttgcacttgccagatatgccgatctgttgaattcacctaaaaagagtgttttacttgctttggctgctcatgcatctgatcccaaagaggccgagcggctcagacatctagcatctcctgctggaaagaaggagtattctcagtggataatcgctagtcaaagaagtctcttggaagttatttcggagtttccatcggcgaaacctccgcttggtgtcttctttgcagctattgctcctcgccttcagccgagatactactcaatatcttcctcaccaagaatggcacctacaagaattcatgtaacatgttcactagttcatgggcaaaccccaactggaaggatccataaaggagtttgttctacttggatgaagaattcaactcccttggaagagagccaagaatgtagctgggctccaatttttgtgaggcagtcaaacttcaaattgcctgctgatcccacagtgcctgttataatggtaggccctgggactggccttgcacctttcaggggcttcttacaggaaagattagctttaaaagagaccggggtggaactgggccgtgccatcctgtttttcgggtgcagaaaccgccagatggacttcatatatgaggatgagctgaacaactttgccgaatccggagccctgtctgagttggtcgtcgccttttctcgtgagggtcctacaaaggagtacgtccaacataaaatggcagagaaggctgcagagctgtggagcattgtttcccagggcggctatgtgtacgtctgcggcgacgccaagggcatggcgagagacgtgcaccgcgcgctgcacaccatagttcaggagcagggatctctggacagctccaaggcggagggctatgtgaaaaaccttcagatggaagggagatacctgagagacgtctggtaa

SEQ ID NO: 22 - DNA, 2112 bp, Triticum aestivum
atggactccgccgccgcggggatgagggactcggcgctcgacctgctggcggcgctgctcacgggccgggccccgccggccgccgccgacggggaccagaaccgccgcctgctcgcgctgctcgccacctccctcgccgtgctcgtcggctgcggcgtcgcgctcctcttccgccgctcctcctccggcgccgcgccgctcgcccacaagtccgccgcggccaagcccctcgcagcgaagaaggaccaggagcccgaccccgacgacggccgccagcgggtcgccctcttcttcggcacgcagaccggcaccgccgagggcttcgccaaggcgctcgcggaggaggccaaggccaggtacgacaaggccgtcttcaaggtgctcgatctggatgactatgccgcggaggacgaggagtacgaggagaagctcaagaaggagaacatcgccttcttcttcctcgcaacgtatggggacggtgagccaaccgacaatgccgccagattctacaaatggttctccgagggaaacgagaggggtgagtggttgagcaacctcaagttcggggtgtttgctcttgggaataggcagtacgagcatttcaacaaggtcggaaaggaggtcgatcagctcctcgccgaacaaggtggaaagcgcatagttcctgttggccttggagatgacgatcaatgcattgaggatgacttcaatgcctggaaggaactactgtggccagaattggacaaactgctccgcgttgaagataattcttcaacagcacaatctccttacacagctgctattccgcaatatagagttgtgcttaccaaaccagaggatgccacacatatcaacaagtctttcagtcttagcaatggtcatgtcgtctacgacagtcaacatccttgcagggcaaatgtggctgtgcgacgggagcttcacacaccagcttctgaccggtcctgcattcatttggaatttgatattgcaggaactagccttacatatgagactggagatcatgttggtgtgtacgcagaaaattcaattgagactgtagaggaggcagaaaagctattagattattcaccagatacttatttctcaatttatgctgaccaagaggatggcactccactttttgggggctctttgccacctcctttcccatctccctgtactgtgagggttgcacttgccagatatgccgatctgttgaattcacctaaaaagagtgttttacttgctttggctgctcatgcatctgatcccaaagaggccgagcggctcagacatctagcatctcctgctggaaagaaggagtattctcagtggataatcgctagtcaaagaagtctcttggaagttatttcggagtttccatcggcgaaacctccgcttggtgtcttctttgcagctattgctcctcgccttcagccgagatactactcaatatcttcctcaccaagaatggcacctacaagaattcatgtaacatgttcactagttcatgggcaaaccccaactggaaggatccataaaggagtttgttctacttggatgaagaattcaactcccttggaagagagccaagaatgtagctgggctccaatttttgtgaggcagtcaaacttcaaattgcctgctgatcccacagtgcctattataatggtaggccctgggactggccttgcacctttcaggggcttcttacaggaaagattagctttaaaagagaccggggtggaactgggccgtgccatcctgtttttcgggtgcagaaaccgccagatggacttcatatatgaggatgagctgaacaactttgccgaatccggagccctgtctgagttggtcgtcgccttttctcgtgagggtcctacaaaggagtacgtccaacataaaatggcagagaaggctgcagagctgtggagcattgtttcccagggcggctatgtgtacgtctgcggcgacgccaagggcatggcgagagacgtgcaccgcgcgctgcacaccatagttcaggagcagggatctctggacagctccaaggcggagggctatgtgaaaaaccttcagatggaagggagatacctgagagacgtctggtaa

SEQ ID NO: 23 - DNA, 21 bp, Artificial
  Synthetic DNA
cacgcgtccgatcgaaccaac

SEQ ID NO: 24 - DNA, 26 bp, Artificial
  Synthetic DNA
cgatgaatcgtcatcctctgttccac

SEQ ID NO: 25 - DNA, 35 bp, Artificial
  Synthetic DNA
aaggagatatacatatggactccgccgccgcgggg

SEQ ID NO: 26 - DNA, 35 bp, Artificial
  Synthetic DNA
ctttaccagactcgattaccagacgtctctcaggt

SEQ ID NO: 27 - DNA, 35 bp, Artificial
  Synthetic DNA
aaggagatatacatatggctaagaagacttcttct

SEQ ID NO: 28 - DNA, 35 bp, Artificial; identical to SEQ ID NO: 20
  Synthetic DNA

SEQ ID NO: 29 - DNA, 35 bp, Artificial
  Synthetic DNA
aaggagatatacatatggaccagaaccgccgcctg

SEQ ID NO: 30 - DNA, 35 bp, Artificial
  Synthetic DNA
tttaccagactcgagttaccagacgtctctcaggt

SEQ ID NO: 31 - DNA, 35 bp, Artificial
  Synthetic DNA
tacaactacatctagaatggataaggcgtacattg

SEQ ID NO: 32 - DNA, 35 bp, Artificial
  Synthetic DNA
ggggaaattcgagctctcagaggctctgaagcacg

SEQ ID NO: 33 - DNA, 22 bp, Artificial
  Synthetic DNA
gctctccaacaacattgccaac

SEQ ID NO: 34 - DNA, 21 bp, Artificial
  Synthetic DNA
gcttctgcctgtcacatacgc

SEQ ID NO: 35 - DNA, 20 bp, Artificial
  Synthetic DNA
ctctgcgcgaatttatttgg

SEQ ID NO: 36 - DNA, 20 bp, Artificial
  Synthetic DNA
tcacgatgcactgcaggtag

SEQ ID NO: 37 - DNA, 23 bp, Artificial
  Synthetic DNA
caacctgagacctcaagtgtcac

SEQ ID NO: 38 - DNA, 23 bp, Artificial
  Synthetic DNA
cagtgctaccgcaagatagctac